European Patent Application EP 4 386 088 A1, published June 19, 2024. Title: Method for the accurate quantification of non-coding RNAs in minute quantities. Applicant: Johannes Gutenberg Universität. Application EP. The sequence listing filed with the application follows.

SEQUENCE LISTING (258 sequences)

SEQ ID NO: 1 - DNA, 21 bp, synthetic construct
  source 1..21: mol_type = other DNA
agacgtgtgctcttccgatct

SEQ ID NO: 2 - DNA, 26 bp, synthetic construct
  source 1..26: mol_type = other DNA
gatcgtcggactgtagaactctgaac

SEQ ID NO: 3 - DNA, 26 bp, synthetic construct
  source 1..26: mol_type = other DNA
gatcgtcggactgtagaactctgaac

SEQ ID NO: 4 - DNA, 63 bp, synthetic construct
  source 1..63: mol_type = other DNA
aatgatacggcgaccaccgagatctacactatagcctgttcagagttctacagtccgacgatc

SEQ ID NO: 5 - DNA, 63 bp, synthetic construct
  source 1..63: mol_type = other DNA
aatgatacggcgaccaccgagatctacacatagaggcgttcagagttctacagtccgacgatc

SEQ ID NO: 6 - DNA, 63 bp, synthetic construct
  source 1..63: mol_type = other DNA
aatgatacggcgaccaccgagatctacaccctatcctgttcagagttctacagtccgacgatc

SEQ ID NO: 7 - DNA, 63 bp, synthetic construct
  source 1..63: mol_type = other DNA
aatgatacggcgaccaccgagatctacacggctctgagttcagagttctacagtccgacgatc

SEQ ID NO: 8 - DNA, 63 bp, synthetic construct
  source 1..63: mol_type = other DNA
aatgatacggcgaccaccgagatctacacaggcgaaggttcagagttctacagtccgacgatc

SEQ ID NO: 9 - DNA, 63 bp, synthetic construct
  source 1..63: mol_type = other DNA
aatgatacggcgaccaccgagatctacactaatcttagttcagagttctacagtccgacgatc

SEQ ID NO: 10 - DNA, 63 bp, synthetic construct
  source 1..63: mol_type = other DNA
aatgatacggcgaccaccgagatctacacacgtcctggttcagagttctacagtccgacgatc

SEQ ID NO: 11 - DNA, 63 bp, synthetic construct
  source 1..63: mol_type = other DNA
aatgatacggcgaccaccgagatctacacgtactgacgttcagagttctacagtccgacgatc

SEQ ID NO: 12 - DNA, 66 bp, synthetic construct
  source 1..66: mol_type = other DNA
caagcagaagacggcatacgagatcgagtaatgtgactggagttcagacgtgtgctcttccgatct

SEQ ID NO: 13 - DNA, 66 bp, synthetic construct
  source 1..66: mol_type = other DNA
caagcagaagacggcatacgagattctccggagtgactggagttcagacgtgtgctcttccgatct

SEQ ID NO: 14 - DNA, 66 bp, synthetic construct
  source 1..66: mol_type = other DNA
caagcagaagacggcatacgagataatgagcggtgactggagttcagacgtgtgctcttccgatct

SEQ ID NO: 15 - DNA, 66 bp, synthetic construct
  source 1..66: mol_type = other DNA
caagcagaagacggcatacgagatggaatctcgtgactggagttcagacgtgtgctcttccgatct

SEQ ID NO: 16 - DNA, 66 bp, synthetic construct
  source 1..66: mol_type = other DNA
caagcagaagacggcatacgagatttctgaatgtgactggagttcagacgtgtgctcttccgatct

SEQ ID NO: 17 - DNA, 66 bp, synthetic construct
  source 1..66: mol_type = other DNA
caagcagaagacggcatacgagatacgaattcgtgactggagttcagacgtgtgctcttccgatct

SEQ ID NO: 18 - DNA, 66 bp, synthetic construct
  source 1..66: mol_type = other DNA
caagcagaagacggcatacgagatagcttcaggtgactggagttcagacgtgtgctcttccgatct

SEQ ID NO: 19 - DNA, 66 bp, synthetic construct
  source 1..66: mol_type = other DNA
caagcagaagacggcatacgagatgcgcattagtgactggagttcagacgtgtgctcttccgatct

SEQ ID NO: 20 - DNA, 66 bp, synthetic construct
  source 1..66: mol_type = other DNA
caagcagaagacggcatacgagatcatagccggtgactggagttcagacgtgtgctcttccgatct

SEQ ID NO: 21 - DNA, 66 bp, synthetic construct
  source 1..66: mol_type = other DNA
caagcagaagacggcatacgagatttcgcggagtgactggagttcagacgtgtgctcttccgatct

SEQ ID NO: 22 - DNA, 66 bp, synthetic construct
  source 1..66: mol_type = other DNA
caagcagaagacggcatacgagatgcgcgagagtgactggagttcagacgtgtgctcttccgatct

SEQ ID NO: 23 - DNA, 66 bp, synthetic construct
  source 1..66: mol_type = other DNA
caagcagaagacggcatacgagatctatcgctgtgactggagttcagacgtgtgctcttccgatct

SEQ ID NO: 24 - DNA, 87 bp, synthetic construct
  source 1..87: mol_type = other DNA
agacgtgtgctcttccgatcttggtggagctaagcgggatcgaaccgcagacctcctgcatgatcgtcggactgtagaactctgaac

SEQ ID NO: 25 - DNA, 87 bp, synthetic construct
  source 1..87: mol_type = other DNA
agacgtgtgctcttccgatcttggtgcatccgggaggattcgaacctccgaccgctcggttgatcgtcggactgtagaactctgaac

SEQ ID NO: 26 - DNA, 87 bp, synthetic construct
  source 1..87: mol_type = other DNA
agacgtgtgctcttccgatcttggcgcgcccgacaggattcgaacctgagacctctgcctcgatcgtcggactgtagaactctgaac

SEQ ID NO: 27 - DNA, 87 bp, synthetic construct
  source 1..87: mol_type = other DNA
agacgtgtgctcttccgatcttggtgtcccctgcaggaatcgaacctgcaattagcccttagatcgtcggactgtagaactctgaac

SEQ ID NO: 28 - DNA, 87 bp, synthetic construct
  source 1..87: mol_type = other DNA
agacgtgtgctcttccgatcttggcgcgccctgcaggattcgaacctgcggcccacgacttgatcgtcggactgtagaactctgaac

SEQ ID NO: 29 - DNA, 87 bp, synthetic construct
  source 1..87: mol_type = other DNA
agacgtgtgctcttccgatcttggctcctctgactggactcgaaccagtgacatacggattgatcgtcggactgtagaactctgaac

SEQ ID NO: 30 - DNA, 87 bp, synthetic construct
  source 1..87: mol_type = other DNA
agacgtgtgctcttccgatcttggcggaacggacgggactcgaacccgcgaccccctgcgtgatcgtcggactgtagaactctgaac

SEQ ID NO: 31 - DNA, 87 bp, synthetic construct
  source 1..87: mol_type = other DNA
agacgtgtgctcttccgatcttggaggcgcgttccggagtcgaaccggactagacggatttgatcgtcggactgtagaactctgaac

SEQ ID NO: 32 - DNA, 87 bp, synthetic construct
  source 1..87: mol_type = other DNA
agacgtgtgctcttccgatcttggttgcgggggccggatttgaaccgacgaccttcgggttgatcgtcggactgtagaactctgaac

SEQ ID NO: 33 - DNA, 87 bp, synthetic construct
  source 1..87: mol_type = other DNA
agacgtgtgctcttccgatcttggctggggtacctggattcgaacctcggaatgccggaatgatcgtcggactgtagaactctgaac

SEQ ID NO: 34 - DNA, 87 bp, synthetic construct
  source 1..87: mol_type = other DNA
agacgtgtgctcttccgatcttggcgtcccctaggggattcgaacccctgttaccgccgtggatcgtcggactgtagaactctgaac

SEQ ID NO: 35 - DNA, 87 bp, synthetic construct
  source 1..87: mol_type = other DNA
agacgtgtgctcttccgatcttggagcgggaaacgagactcgaactcgcgaccccgaccttgatcgtcggactgtagaactctgaac

SEQ ID NO: 36 - DNA, 87 bp, synthetic construct
  source 1..87: mol_type = other DNA
agacgtgtgctcttccgatcttggagcgggcgaagggaatcgaaccctcgtatagagcttggatcgtcggactgtagaactctgaac

SEQ ID NO: 37 - DNA, 87 bp, synthetic construct
  source 1..87: mol_type = other DNA
agacgtgtgctcttccgatcttggagcgggcagcgggaatcgaacccgcatcatcagcttggatcgtcggactgtagaactctgaac

SEQ ID NO: 38 - DNA, 87 bp, synthetic construct
  source 1..87: mol_type = other DNA
agacgtgtgctcttccgatcttggggtggctaatgggattcgaacccacgacaactggaatgatcgtcggactgtagaactctgaac

SEQ ID NO: 39 - DNA, 87 bp, synthetic construct
  source 1..87: mol_type = other DNA
agacgtgtgctcttccgatcttggtaggcctgagtggacttgaaccaccgacctcacccttgatcgtcggactgtagaactctgaac

SEQ ID NO: 40 - DNA, 87 bp, synthetic construct
  source 1..87: mol_type = other DNA
agacgtgtgctcttccgatcttggtggcccttgctggacttgaaccagcgaccaagcgattgatcgtcggactgtagaactctgaac

SEQ ID NO: 41 - DNA, 87 bp, synthetic construct
  source 1..87: mol_type = other DNA
agacgtgtgctcttccgatcttggtgcgaggggggggacttgaacccccacgtccgtaagggatcgtcggactgtagaactctgaac

SEQ ID NO: 42 - DNA, 87 bp, synthetic construct
  source 1..87: mol_type = other DNA
agacgtgtgctcttccgatcttggtgccgaaggccggactcgaaccggcacgtatttctacgatcgtcggactgtagaactctgaac

SEQ ID NO: 43 - DNA, 87 bp, synthetic construct
  source 1..87: mol_type = other DNA
agacgtgtgctcttccgatcttggtaccgaggacgggacttgaacccgtaagccctattgggatcgtcggactgtagaactctgaac

SEQ ID NO: 44 - DNA, 87 bp, synthetic construct
  source 1..87: mol_type = other DNA
agacgtgtgctcttccgatcttggtacccggagcgggacttgaacccgcacagcgcgaacggatcgtcggactgtagaactctgaac

SEQ ID NO: 45 - DNA, 87 bp, synthetic construct
  source 1..87: mol_type = other DNA
agacgtgtgctcttccgatcttggtgcgggaggcgagacttgaactcgcacaccttgcggcgatcgtcggactgtagaactctgaac

SEQ ID NO: 46 - DNA, 87 bp, synthetic construct
  source 1..87: mol_type = other DNA
agacgtgtgctcttccgatcttggtgggtcgtgcaggattcgaacctgcgaccaattgattgatcgtcggactgtagaactctgaac

SEQ ID NO: 47 - DNA, 87 bp, synthetic construct
  source 1..87: mol_type = other DNA
agacgtgtgctcttccgatcttggtggctacgacgggattcgaacctgtgaccccatcattgatcgtcggactgtagaactctgaac

SEQ ID NO: 48 - DNA, 87 bp, synthetic construct
  source 1..87: mol_type = other DNA
agacgtgtgctcttccgatcttggtgcccggactcggaatcgaaccaaggacacggggattgatcgtcggactgtagaactctgaac

SEQ ID NO: 49 - DNA, 87 bp, synthetic construct
  source 1..87: mol_type = other DNA
agacgtgtgctcttccgatcttggtcggtgatagaggattcgaacctccgaccccttcgtcgatcgtcggactgtagaactctgaac

SEQ ID NO: 50 - DNA, 87 bp, synthetic construct
  source 1..87: mol_type = other DNA
agacgtgtgctcttccgatcttggtcggcacgagaggatttgaacctccgacccccgacacgatcgtcggactgtagaactctgaac

SEQ ID NO: 51 - DNA, 87 bp, synthetic construct
  source 1..87: mol_type = other DNA
agacgtgtgctcttccgatcttggtcggcgagagaggattcgaacctccgacccactggtcgatcgtcggactgtagaactctgaac

SEQ ID NO: 52 - DNA, 87 bp, synthetic construct
  source 1..87: mol_type = other DNA
agacgtgtgctcttccgatcttggcggaagatcacaggagtcgaacctgcccgggaccgctgatcgtcggactgtagaactctgaac

SEQ ID NO: 53 - DNA, 87 bp, synthetic construct
  source 1..87: mol_type = other DNA
agacgtgtgctcttccgatcttggcggtgagggggggattcgaacccccgatacgttgccggatcgtcggactgtagaactctgaac

SEQ ID NO: 54 - DNA, 87 bp, synthetic construct
  source 1..87: mol_type = other DNA
agacgtgtgctcttccgatcttggcggagagagggggatttgaacccccggtagagttgccgatcgtcggactgtagaactctgaac

SEQ ID NO: 55 - DNA, 87 bp, synthetic construct
  source 1..87: mol_type = other DNA
agacgtgtgctcttccgatcttggcggtgaggcggggattcgaaccccggatgcagcttttgatcgtcggactgtagaactctgaac

SEQ ID NO: 56 - DNA, 87 bp, synthetic construct
  source 1..87: mol_type = other DNA
agacgtgtgctcttccgatcttggcggaagcgcagagattcgaactctggaaccctttcgggatcgtcggactgtagaactctgaac

SEQ ID NO: 57 - DNA, 87 bp, synthetic construct
  source 1..87: mol_type = other DNA
agacgtgtgctcttccgatcttggtgccgataataggagtcgaacctacgaccttcgcattgatcgtcggactgtagaactctgaac

SEQ ID NO: 58 - DNA, 87 bp, synthetic construct
  source 1..87: mol_type = other DNA
agacgtgtgctcttccgatcttggtgctgatacccagagtcgaactgccgacctcacccttgatcgtcggactgtagaactctgaac

SEQ ID NO: 59 - DNA, 87 bp, synthetic construct
  source 1..87: mol_type = other DNA
agacgtgtgctcttccgatcttggtgccgactaccggaatcgaactggtgacctactgattgatcgtcggactgtagaactctgaac

SEQ ID NO: 60 - DNA, 87 bp, synthetic construct
  source 1..87: mol_type = other DNA
agacgtgtgctcttccgatcttggcaggggcggagagactcgaactcccaacacccggtttgatcgtcggactgtagaactctgaac

SEQ ID NO: 61 - DNA, 87 bp, synthetic construct
  source 1..87: mol_type = other DNA
agacgtgtgctcttccgatcttggtggtgggggaaggattcgaaccttcgaagtcgatgacgatcgtcggactgtagaactctgaac

SEQ ID NO: 62 - DNA, 87 bp, synthetic construct
  source 1..87: mol_type = other DNA
agacgtgtgctcttccgatcttggtgggtgatgacgggatcgaaccgccgaccccctccttgatcgtcggactgtagaactctgaac

SEQ ID NO: 63 - DNA, 87 bp, synthetic construct
  source 1..87: mol_type = other DNA
agacgtgtgctcttccgatcttggtgcgtccgagtggactcgaaccaacgacccccaccatgatcgtcggactgtagaactctgaac

SEQ ID NO: 64 - DNA, 87 bp, synthetic construct
  source 1..87: mol_type = other DNA
agacgtgtgctcttccgatcttggtggagttaatgagacttgaactcatattaaatgcatggatcgtcggactgtagaactctgaac

SEQ ID NO: 65 - DNA, 87 bp, synthetic construct
  source 1..87: mol_type = other DNA
agacgtgtgctcttccgatcttggaatatcttataggatttgaacctatataattagattcgatcgtcggactgtagaactctgaac

SEQ ID NO: 66 - DNA, 87 bp, synthetic construct
  source 1..87: mol_type = other DNA
agacgtgtgctcttccgatcttggtactctctccatgatttgaacatggaatattaatattgatcgtcggactgtagaactctgaac

SEQ ID NO: 67 - DNA, 87 bp, synthetic construct
  source 1..87: mol_type = other DNA
agacgtgtgctcttccgatcttggcgtccttaataggaattgaacccatctattctcattagatcgtcggactgtagaactctgaac

SEQ ID NO: 68 - DNA, 87 bp, synthetic construct
  source 1..87: mol_type = other DNA
agacgtgtgctcttccgatcttggcgaatctaatcagatttgcactgacatcctccattatgatcgtcggactgtagaactctgaac

SEQ ID NO: 69 - DNA, 87 bp, synthetic construct
  source 1..87: mol_type = other DNA
agacgtgtgctcttccgatcttggaagagatgaagagaatcgaactcttaataagtagattgatcgtcggactgtagaactctgaac

SEQ ID NO: 70 - DNA, 87 bp, synthetic construct
  source 1..87: mol_type = other DNA
agacgtgtgctcttccgatcttggtagcaataatacgatttgaacgtatataattaggtcagatcgtcggactgtagaactctgaac

SEQ ID NO: 71 - DNA, 87 bp, synthetic construct
  source 1..87: mol_type = other DNA
agacgtgtgctcttccgatcttggttgaatcgctttgattcgaacaaagaactccaaactcgatcgtcggactgtagaactctgaac

SEQ ID NO: 72 - DNA, 87 bp, synthetic construct
  source 1..87: mol_type = other DNA
agacgtgtgctcttccgatcttggtaaccttaatcggaatcgaaccgatattatcaacatggatcgtcggactgtagaactctgaac

SEQ ID NO: 73 - DNA, 87 bp, synthetic construct
  source 1..87: mol_type = other DNA
agacgtgtgctcttccgatcttggtatagatagcgagaatcgaactcgcattcaatgtttggatcgtcggactgtagaactctgaac

SEQ ID NO: 74 - DNA, 87 bp, synthetic construct
  source 1..87: mol_type = other DNA
agacgtgtgctcttccgatcttggggtgaatactgagaatcgaactcagatttaacgcaccgatcgtcggactgtagaactctgaac

SEQ ID NO: 75 - DNA, 87 bp, synthetic construct
  source 1..87: mol_type = other DNA
agacgtgtgctcttccgatcttggtgaaactaacagggattgaacctatatttgtaccttagatcgtcggactgtagaactctgaac

SEQ ID NO: 76 - DNA, 87 bp, synthetic construct
  source 1..87: mol_type = other DNA
agacgtgtgctcttccgatcttggtgctatttaaaggacttgaaccttcatactgtaaagtgatcgtcggactgtagaactctgaac

SEQ ID NO: 77 - DNA, 87 bp, synthetic construct
  source 1..87: mol_type = other DNA
agacgtgtgctcttccgatcttggtgagaatagctggagttgaacctgcatgggttgcttagatcgtcggactgtagaactctgaac

SEQ ID NO: 78 - DNA, 87 bp, synthetic construct
  source 1..87: mol_type = other DNA
agacgtgtgctcttccgatcttggtacttgtagaaggaattgaaccttacattatttatttgatcgtcggactgtagaactctgaac

SEQ ID NO: 79 - DNA, 87 bp, synthetic construct
  source 1..87: mol_type = other DNA
agacgtgtgctcttccgatcttggtgcccttaatgagaatcgaacttatgtaaataaatctgatcgtcggactgtagaactctgaac

SEQ ID NO: 80 - DNA, 87 bp, synthetic construct
  source 1..87: mol_type = other DNA
agacgtgtgctcttccgatcttggtcagataggatagactcgaactaactaggtctttctcgatcgtcggactgtagaactctgaac

SEQ ID NO: 81 - DNA, 87 bp, synthetic construct
  source 1..87: mol_type = other DNA
agacgtgtgctcttccgatcttggcggaaaatatgagattcgaactcataagaatttacaagatcgtcggactgtagaactctgaac

SEQ ID NO: 82 - DNA, 87 bp, synthetic construct
  source 1..87: mol_type = other DNA
agacgtgtgctcttccgatcttggcggatgatgtaggatttgaacctacgtagccaataaagatcgtcggactgtagaactctgaac

SEQ ID NO: 83 - DNA, 87 bp, synthetic construct
  source 1..87: mol_type = other DNA
agacgtgtgctcttccgatcttggtgtaaatactaagatttgaacttagataatatgcaccgatcgtcggactgtagaactctgaac

SEQ ID NO: 84 - DNA, 87 bp, synthetic construct
  source 1..87: mol_type = other DNA
agacgtgtgctcttccgatcttggtgttatattagggatttgaaccccaaacctttcgattgatcgtcggactgtagaactctgaac

SEQ ID NO: 85 - DNA, 87 bp, synthetic construct
  source 1..87: mol_type = other DNA
agacgtgtgctcttccgatcttggcaaggataaagagattcgaactcctaatgattgatttgatcgtcggactgtagaactctgaac

SEQ ID NO: 86 - DNA, 87 bp, synthetic construct
  source 1..87: mol_type = other DNA
agacgtgtgctcttccgatcttggtaaagggaataggaattgaacctatgaagacctaagtgatcgtcggactgtagaactctgaac

SEQ ID NO: 87 - DNA, 87 bp, synthetic construct
  source 1..87: mol_type = other DNA
agacgtgtgctcttccgatcttggtaggaaatatagggttcgaacctataatctttcgtgtgatcgtcggactgtagaactctgaac

SEQ ID NO: 88 - DNA, 87 bp, synthetic construct
  source 1..87: mol_type = other DNA
agacgtgtgctcttccgatcttggtggacgagtccggaatcgaaccggagacctctcccacgatcgtcggactgtagaactctgaac

SEQ ID NO: 89 - DNA, 87 bp, synthetic construct
  source 1..87: mol_type = other DNA
agacgtgtgctcttccgatcttgggtggacgcaaccggaatcgaaccgatgacctcttcctgatcgtcggactgtagaactctgaac

SEQ ID NO: 90 - DNA, 87 bp, synthetic construct
  source 1..87: mol_type = other DNA
agacgtgtgctcttccgatcttggcactcacgatgggggtcgaacccataatcttctgattgatcgtcggactgtagaactctgaac

SEQ ID NO: 91 - DNA, 87 bp, synthetic construct
  source 1..87: mol_type = other DNA
agacgtgtgctcttccgatcttggagctcctcccgggactcgaacccggatcacagccaccgatcgtcggactgtagaactctgaac

SEQ ID NO: 92 - DNA, 87 bp, synthetic construct
  source 1..87: mol_type = other DNA
agacgtgtgctcttccgatcttggcgttccgtacgggactcgaacccgcagtcttctccttgatcgtcggactgtagaactctgaac

SEQ ID NO: 93 - DNA, 87 bp, synthetic construct
  source 1..87: mol_type = other DNA
agacgtgtgctcttccgatcttggcttccccgccaggacttgaacctggaatcttctggttgatcgtcggactgtagaactctgaac

SEQ ID NO: 94 - DNA, 87 bp, synthetic construct
  source 1..87: mol_type = other DNA
agacgtgtgctcttccgatcttggcgaccccagtgagggttgaactcacgatcttgcgattgatcgtcggactgtagaactctgaac

SEQ ID NO: 95 - DNA, 87 bp, synthetic construct
  source 1..87: mol_type = other DNA
agacgtgtgctcttccgatcttggctccgcgacggggaattgaaccccgatctggcacgcggatcgtcggactgtagaactctgaac

SEQ ID NO: 96 - DNA, 87 bp, synthetic construct
  source 1..87: mol_type = other DNA
agacgtgtgctcttccgatcttggagctcgcactcaggatcgaactaaggaccaacagattgatcgtcggactgtagaactctgaac

SEQ ID NO: 97 - DNA, 87 bp, synthetic construct
  source 1..87: mol_type = other DNA
agacgtgtgctcttccgatcttggtagcgccgctcggtttcgatccgaggacatcagggttgatcgtcggactgtagaactctgaac

SEQ ID NO: 98 - DNA, 87 bp, synthetic construct
  source 1..87: mol_type = other DNA
agacgtgtgctcttccgatcttggtcttacccggattcgaaccggggttgttcggatcaaagatcgtcggactgtagaactctgaac

SEQ ID NO: 99 - DNA, 87 bp, synthetic construct
  source 1..87: mol_type = other DNA
agacgtgtgctcttccgatcttggctccgatacggggagtcgaaccccggtctccacggtggatcgtcggactgtagaactctgaac

SEQ ID NO: 100 - DNA, 87 bp, synthetic construct
  source 1..87: mol_type = other DNA
agacgtgtgctcttccgatcttggtgagcggtacgagaatcgaacccgtgtccccaccttggatcgtcggactgtagaactctgaac

SEQ ID NO: 101 - DNA, 87 bp, synthetic construct
  source 1..87: mol_type = other DNA
agacgtgtgctcttccgatcttggtgcggaagccgggaatcgaacccgggccccatgcttggatcgtcggactgtagaactctgaac

SEQ ID NO: 102 - DNA, 87 bp, synthetic construct
  source 1..87: mol_type = other DNA
agacgtgtgctcttccgatcttggtgcgcaagcccggaatcgaaccggggcccaacgatgggatcgtcggactgtagaactctgaac

SEQ ID NO: 103 - DNA, 87 bp, synthetic construct
  source 1..87: mol_type = other DNA
agacgtgtgctcttccgatcttggtgccacctcctagaatcgaaccagggtttcaacagccgatcgtcggactgtagaactctgaac

SEQ ID NO: 104 - DNA, 87 bp, synthetic construct
  source 1..87: mol_type = other DNA
agacgtgtgctcttccgatcttggtggtctctagcgggatcgaaccgcttatccccgcgttgatcgtcggactgtagaactctgaac

SEQ ID NO: 105 - DNA, 87 bp, synthetic construct
  source 1..87: mol_type = other DNA
agacgtgtgctcttccgatcttggtgctcgaggtggggtttgaacccacgacggtcgcgttgatcgtcggactgtagaactctgaac

SEQ ID NO: 106 - DNA, 87 bp, synthetic construct
  source 1..87: mol_type = other DNA
agacgtgtgctcttccgatcttggtgatacccgcggggtttgaacccgcgcctccgaagaggatcgtcggactgtagaactctgaac

SEQ ID NO: 107 - DNA, 87 bp, synthetic construct
  source 1..87: mol_type = other DNA
agacgtgtgctcttccgatcttggtgaaggatgcgaggttcgaactcgcgcggacaaccgtgatcgtcggactgtagaactctgaac

SEQ ID NO: 108 - DNA, 87 bp, synthetic construct
  source 1..87: mol_type = other DNA
agacgtgtgctcttccgatcttggtggttgctaagagattcgaactcttgcatcttacgatgatcgtcggactgtagaactctgaac

SEQ ID NO: 109 - DNA, 87 bp, synthetic construct
  source 1..87: mol_type = other DNA
agacgtgtgctcttccgatcttggctcctcatagggggctcgaacccctgacatttcggttgatcgtcggactgtagaactctgaac

SEQ ID NO: 110 - DNA, 87 bp, synthetic construct
  source 1..87: mol_type = other DNA
agacgtgtgctcttccgatcttggtgctccaggagaggttcgaactctcgaccttcagattgatcgtcggactgtagaactctgaac

SEQ ID NO: 111 - DNA, 87 bp, synthetic construct
  source 1..87: mol_type = other DNA
agacgtgtgctcttccgatcttggtgcgaattctgtggatcgaacacaggacctccagatcgatcgtcggactgtagaactctgaac

SEQ ID NO: 112 - DNA, 87 bp, synthetic construct
  source 1..87: mol_type = other DNA
agacgtgtgctcttccgatctatggtgttccaaccgaggatcgaactcgggacctttgccggatcgtcggactgtagaactctgaac

SEQ ID NO: 113 - DNA, 87 bp, synthetic construct
  source 1..87: mol_type = other DNA
agacgtgtgctcttccgatcttggggggcgagctgggaattgaacccagggcctctcgcacgatcgtcggactgtagaactctgaac

SEQ ID NO: 114 - DNA, 87 bp, synthetic construct
  source 1..87: mol_type = other DNA
agacgtgtgctcttccgatcttggcgtcacagacaggattcgaacctgcgcaggtaaaaccgatcgtcggactgtagaactctgaac

SEQ ID NO: 115 - DNA, 87 bp, synthetic construct
  source 1..87: mol_type = other DNA
agacgtgtgctcttccgatcttggcgacaactgcaggactcgaacctgcgcgggcaaagccgatcgtcggactgtagaactctgaac

SEQ ID NO: 116 - DNA, 87 bp, synthetic construct
  source 1..87: mol_type = other DNA
agacgtgtgctcttccgatcttggcgacaccagcaggatttgaaccagcgcgggcagagccgatcgtcggactgtagaactctgaac

SEQ ID NO: 117 - DNA, 87 bp, synthetic construct
  source 1..87: mol_type = other DNA
agacgtgtgctcttccgatctatggcgacaccagcaggatttgaaccagcgcgggcagagcgatcgtcggactgtagaactctgaac

SEQ ID NO: 118 - DNA, 87 bp, synthetic construct
  source 1..87: mol_type = other DNA
agacgtgtgctcttccgatcttggtgccctctgtgggaattgaacccacgatccccgcattgatcgtcggactgtagaactctgaac

SEQ ID NO: 119 - DNA, 87 bp, synthetic construct
  source 1..87: mol_type = other DNA
agacgtgtgctcttccgatcttggtgcttccaatcggatttgaaccgatgatctccacattgatcgtcggactgtagaactctgaac

SEQ ID NO: 120 - DNA, 87 bp, synthetic construct
  source 1..87: mol_type = other DNA
agacgtgtgctcttccgatcttggtgccacctgtcagaattgaactaacgacctttgcattgatcgtcggactgtagaactctgaac

SEQ ID NO: 121 - DNA, 87 bp, synthetic construct
  source 1..87: mol_type = other DNA
agacgtgtgctcttccgatcttggtgaaacggacaggaattgaacctgcaacccttcgattgatcgtcggactgtagaactctgaac

SEQ ID NO: 122 - DNA, 87 bp, synthetic construct
  source 1..87: mol_type = other DNA
agacgtgtgctcttccgatcttggtctcccgggggcgagtcgaacgcccgatctcaagattgatcgtcggactgtagaactctgaac

SEQ ID NO: 123 - DNA, 87 bp, synthetic construct
  source 1..87: mol_type = other DNA
agacgtgtgctcttccgatcttggggggcgagccgggactcgaacccgggacctcccgcaggatcgtcggactgtagaactctgaac

SEQ ID NO: 124 - DNA, 87 bp, synthetic construct
  source 1..87: mol_type = other DNA
agacgtgtgctcttccgatcttggtgatttcgcccaggatcgaactggggacgttctgcgtgatcgtcggactgtagaactctgaac

SEQ ID NO: 125 - DNA, 87 bp, synthetic construct
  source 1..87: mol_type = other DNA
agacgtgtgctcttccgatcttggtgatccaaccgaggttcgaactcgggatcttcgccgtgatcgtcggactgtagaactctgaac

SEQ ID NO: 126 - DNA, 87 bp, synthetic construct
  source 1..87: mol_type = other DNA
agacgtgtgctcttccgatcttggtaaggactgcaaaaccccactctgcatcaactgaacggatcgtcggactgtagaactctgaac

SEQ ID NO: 127 - DNA, 87 bp, synthetic construct
  source 1..87: mol_type = other DNA
agacgtgtgctcttccgatcttggttggtaaatatgattatcataatttaatgagtcgaaagatcgtcggactgtagaactctgaac

SEQ ID NO: 128 - DNA, 87 bp, synthetic construct
  source 1..87: mol_type = other DNA
agacgtgtgctcttccgatcttggctagaccaatgggacttaaacccacaaacacttagttgatcgtcggactgtagaactctgaac

SEQ ID NO: 129 - DNA, 87 bp, synthetic construct
  source 1..87: mol_type = other DNA
agacgtgtgctcttccgatcttggtaagatatataggatttagcctataatttaactttgagatcgtcggactgtagaactctgaac

SEQ ID NO: 130 - DNA, 87 bp, synthetic construct
  source 1..87: mol_type = other DNA
agacgtgtgctcttccgatcttggaagccccggcaggtttgaagctgcttcttcgaatttggatcgtcggactgtagaactctgaac

SEQ ID NO: 131 - DNA, 87 bp, synthetic construct
  source 1..87: mol_type = other DNA
agacgtgtgctcttccgatcttggctaggactatgagaatcgaacccatccctgagaatccgatcgtcggactgtagaactctgaac

SEQ ID NO: 132 - DNA, 87 bp, synthetic construct
  source 1..87: mol_type = other DNA
agacgtgtgctcttccgatcttggtattctcgcacggactacaaccacgaccaatgatatggatcgtcggactgtagaactctgaac

SEQ ID NO: 133 - DNA, 87 bp, synthetic construct
  source 1..87: mol_type = other DNA
agacgtgtgctcttccgatcttggtactcttttttgaatgttgtcaaaactagttaattgggatcgtcggactgtagaactctgaac

SEQ ID NO: 134 - DNA, 87 bp, synthetic construct
  source 1..87: mol_type = other DNA
agacgtgtgctcttccgatcttggggtaaataaggggtcgtaagcctctgttgtcagattcgatcgtcggactgtagaactctgaac

SEQ ID NO: 135 - DNA, 87 bp, synthetic construct
  source 1..87: mol_type = other DNA
agacgtgtgctcttccgatcttggtagaaataagggggtttaagctcctattatttactctgatcgtcggactgtagaactctgaac

SEQ ID NO: 136 - DNA, 87 bp, synthetic construct
  source 1..87: mol_type = other DNA
agacgtgtgctcttccgatcttggtgttaagaagaggaattgaacctctgactgtaaagttgatcgtcggactgtagaactctgaac

SEQ ID NO: 137 - DNA, 87 bp, synthetic construct
  source 1..87: mol_type = other DNA
agacgtgtgctcttccgatcttggtacttttatttggagttgcaccaaaatttttggggccgatcgtcggactgtagaactctgaac

SEQ ID NO: 138 - DNA, 87 bp, synthetic construct
  source 1..87: mol_type = other DNA
agacgtgtgctcttccgatcttggtcactgtaaagaggtgttggttctcttaatctttaacgatcgtcggactgtagaactctgaac

SEQ ID NO: 139 - DNA, 87 bp, synthetic construct
  source 1..87: mol_type = other DNA
agacgtgtgctcttccgatcttggtagtacgggaagggtataaccaacattttcggggtatgatcgtcggactgtagaactctgaac

SEQ ID NO: 140 - DNA, 87 bp, synthetic construct
  source 1..87: mol_type = other DNA
agacgtgtgctcttccgatcttggtgtttatggggtgatgtgagcccgtctaaacattttcgatcgtcggactgtagaactctgaac

SEQ ID NO: 141 - DNA, 87 bp, synthetic construct
  source 1..87: mol_type = other DNA
agacgtgtgctcttccgatcttggtcagagaaaaagtctttaactccaccattagcacccagatcgtcggactgtagaactctgaac

SEQ ID NO: 142 - DNA, 87 bp, synthetic construct
  source 1..87: mol_type = other DNA
agacgtgtgctcttccgatcttggtgagaaagccatgttgttagacatgggggcatgagttgatcgtcggactgtagaactctgaac

SEQ ID NO: 143 - DNA, 87 bp, synthetic construct
  source 1..87: mol_type = other DNA
agacgtgtgctcttccgatcttggcaaaaaaggaaggaatcgaaccccccaaagctggtttgatcgtcggactgtagaactctgaac

SEQ ID NO: 144 - DNA, 87 bp, synthetic construct
  source 1..87: mol_type = other DNA
agacgtgtgctcttccgatcttggtgtccttggaaaaaggttttcatctccggtttacaaggatcgtcggactgtagaactctgaac

SEQ ID NO: 145 - DNA, 87 bp, synthetic construct
  source 1..87: mol_type = other DNA
agacgtgtgctcttccgatcttggcagaaattaagtattgcaacttactgagggctttgaagatcgtcggactgtagaactctgaac

SEQ ID NO: 146 - DNA, 87 bp, synthetic construct
  source 1..87: mol_type = other DNA
agacgtgtgctcttccgatcttggggtaaaaagaggcctaacccctgtctttagatttacagatcgtcggactgtagaactctgaac

SEQ ID NO: 147 - DNA, 87 bp, synthetic construct
  source 1..87: mol_type = other DNA
agacgtgtgctcttccgatcttggtcagagcggtcaagttaagttgaaatctcctaagtgtgatcgtcggactgtagaactctgaac

SEQ ID NO: 148 - DNA, 87 bp, synthetic construct
  source 1..87: mol_type = other DNA
agacgtgtgctcttccgatcttggtggagaatgcgggcatcgatcccgctacctctcgcatgatcgtcggactgtagaactctgaac

SEQ ID NO: 149 - DNA, 87 bp, synthetic construct
  source 1..87: mol_type = other DNA
agacgtgtgctcttccgatcttggtggaggtgccggggatcgaacccggggcctcatacatgatcgtcggactgtagaactctgaac

SEQ ID NO: 150 - DNA, 87 bp, synthetic construct
  source 1..87: mol_type = other DNA
agacgtgtgctcttccgatcttggcgagccagccaggagtcgaacctagaatcttctgatcgatcgtcggactgtagaactctgaac

SEQ ID NO: 151 - DNA, 87 bp, synthetic construct
  source 1..87: mol_type = other DNA
agacgtgtgctcttccgatcttggcgaccacgaagggactcgaaccctcaatcttctgatcgatcgtcggactgtagaactctgaac

SEQ ID NO: 152 - DNA, 87 bp, synthetic construct
  source 1..87: mol_type = other DNA
agacgtgtgctcttccgatcttggcaccccaggtgggactcgaacccacaatccctggcttgatcgtcggactgtagaactctgaac

SEQ ID NO: 153 - DNA, 87 bp, synthetic construct
  source 1..87: mol_type = other DNA
agacgtgtgctcttccgatcttggcgaccgcggcaggactcgaacctgcaatcttctgatcgatcgtcggactgtagaactctgaac

SEQ ID NO: 154 - DNA, 87 bp, synthetic construct
  source 1..87: mol_type = other DNA
agacgtgtgctcttccgatcttggcgactctgccgggactcgaacccgcaacctttgaattgatcgtcggactgtagaactctgaac

SEQ ID NO: 155 - DNA, 87 bp, synthetic construct
  source 1..87: mol_type = other DNA
agacgtgtgctcttccgatcttggcgtccctgggtgggctcgaaccaccaacctttcggttgatcgtcggactgtagaactctgaac

SEQ ID NO: 156 - DNA, 87 bp, synthetic construct
  source 1..87: mol_type = other DNA
agacgtgtgctcttccgatcttggctccccgtcggggaatcgaaccccggtctcccgcgtggatcgtcggactgtagaactctgaac

SEQ ID NO: 157 - DNA, 87 bp, synthetic construct
  source 1..87: mol_type = other DNA
agacgtgtgctcttccgatcttggagggggcacccggatttgaaccagggacctcttgatcgatcgtcggactgtagaactctgaac

SEQ ID NO: 158 - DNA, 87 bp, synthetic construct
  source 1..87: mol_type = other DNA
agacgtgtgctcttccgatcttggtagcagaggatggtttcgatccatcgacctctgggttgatcgtcggactgtagaactctgaac

SEQ ID NO: 159 - DNA, 87 bp, synthetic construct
  source 1..87: mol_type = other DNA
agacgtgtgctcttccgatcttggaggttccaccgagatttgaactcggatcgctggattcgatcgtcggactgtagaactctgaac

SEQ ID NO: 160 - DNA, 87 bp, synthetic construct
  source 1..87: mol_type = other DNA
agacgtgtgctcttccgatcttggttccctgaccgggaatcgaacccgggccgcggcggtggatcgtcggactgtagaactctgaac

SEQ ID NO: 161 - DNA, 87 bp, synthetic construct
  source 1..87: mol_type = other DNA
agacgtgtgctcttccgatcttggttcccacaccgggagtcgaacccgggccgcctgggtggatcgtcggactgtagaactctgaac

SEQ ID NO: 162 - DNA, 87 bp, synthetic construct
  source 1..87: mol_type = other DNA
agacgtgtgctcttccgatcttggtgcgccgcccgggaatcgaacccgggtcgcaagaatggatcgtcggactgtagaactctgaac

SEQ ID NO: 163 - DNA, 87 bp, synthetic construct
  source 1..87: mol_type = other DNA
agacgtgtgctcttccgatcttggtgcattggccgggaatcgaacccgggcctcccgcgtggatcgtcggactgtagaactctgaac

SEQ ID NO: 164 - DNA, 87 bp, synthetic construct
  source 1..87: mol_type = other DNA
agacgtgtgctcttccgatcttggtgcgttggccgggaatcgaacccgggtcaactgcttggatcgtcggactgtagaactctgaac

SEQ ID NO: 165 - DNA, 87 bp, synthetic construct
  source 1..87: mol_type = other DNA
agacgtgtgctcttccgatcttggtgccgtgactcggattcgaaccgaggttgctgcggccgatcgtcggactgtagaactctgaac

SEQ ID NO: 166 - DNA, 87 bp, synthetic construct
  source 1..87: mol_type = other DNA
agacgtgtgctcttccgatcttggtggcccgtacggggatcgaacccgcgaccttggcgttgatcgtcggactgtagaactctgaac

SEQ ID NO: 167 - DNA, 87 bp, synthetic construct
  source 1..87: mol_type = other DNA
agacgtgtgctcttccgatcttggtgctccaggtgaggctcgaactcacaacctcggcattgatcgtcggactgtagaactctgaac

SEQ ID NO: 168 - DNA, 87 bp, synthetic construct
  source 1..87: mol_type = other DNA
agacgtgtgctcttccgatcttggtggcagcggtgggattcgaacccacgcccccgaagaggatcgtcggactgtagaactctgaac

SEQ ID NO: 169 - DNA, 87 bp, synthetic construct
  source 1..87: mol_type = other DNA
agacgtgtgctcttccgatcttggtgccccctctgaggcttgaactcaggaccattcagatgatcgtcggactgtagaactctgaac

SEQ ID NO: 170 - DNA, 87 bp, synthetic construct
  source 1..87: mol_type = other DNA
agacgtgtgctcttccgatcttggtgtcagaagtgggattcgaacccacgcctccatcggagatcgtcggactgtagaactctgaac

SEQ ID NO: 171 - DNA, 87 bp, synthetic construct
  source 1..87: mol_type = other DNA
agacgtgtgctcttccgatcttggtaccaggagtggggttcgaacccacgcggacaccagtgatcgtcggactgtagaactctgaac

SEQ ID NO: 172 - DNA, 87 bp, synthetic construct
  source 1..87: mol_type = other DNA
agacgtgtgctcttccgatcttggcgcccaacgtggggctcgaacccacgaccctgagattgatcgtcggactgtagaactctgaac

SEQ ID NO: 173 - DNA, 87 bp, synthetic construct
  source 1..87: mol_type = other DNA
agacgtgtgctcttccgatcttggcgcctgaacagggacttgaaccctggaccctcagattgatcgtcggactgtagaactctgaac

SEQ ID NO: 174 - DNA, 87 bp, synthetic construct
  source 1..87: mol_type = other DNA
agacgtgtgctcttccgatcttggtgccctctctgaggctcgaactcaggaccttcagattgatcgtcggactgtagaactctgaac

SEQ ID NO: 175 - DNA, 87 bp, synthetic construct
  source 1..87: mol_type = other DNA
agacgtgtgctcttccgatcttggtgccgaaacccgggattgaaccagggacctttagatcgatcgtcggactgtagaactctgaac

SEQ ID NO: 176 - DNA, 87 bp, synthetic construct
  source 1..87: mol_type = other DNA
agacgtgtgctcttccgatcttgggggctcgtccgggatttgaacccgggacctctcgcacgatcgtcggactgtagaactctgaac

SEQ ID NO: 177 - DNA, 87 bp, synthetic construct
  source 1..87: mol_type = other DNA
agacgtgtgctcttccgatcttggcgcccgaaaggtggaattgaaccactctgtcgctagagatcgtcggactgtagaactctgaac

SEQ ID NO: 178 - DNA, 87 bp, synthetic construct
  source 1..87: mol_type = other DNA
agacgtgtgctcttccgatcttggcgtagtcggcaggattcgaacctgcgcggggagacccgatcgtcggactgtagaactctgaac

SEQ ID NO: 179 - DNA, 87 bp, synthetic construct
  source 1..87: mol_type = other DNA
agacgtgtgctcttccgatcttggcgctgtgagcaggatttgaacctgcgcggggagacccgatcgtcggactgtagaactctgaac

SEQ ID NO: 180 - DNA, 87 bp, synthetic construct
  source 1..87: mol_type = other DNA
agacgtgtgctcttccgatcttggcgtcacgaacaggattcgaacctgtgcggggaaacccgatcgtcggactgtagaactctgaac

SEQ ID NO: 181 - DNA, 87 bp, synthetic construct
  source 1..87: mol_type = other DNA
agacgtgtgctcttccgatcttggcgacgaggatgggattcgaacccacgcgtgcagagcagatcgtcggactgtagaactctgaac

SEQ ID NO: 182 - DNA, 87 bp, synthetic construct
  source 1..87: mol_type = other DNA
agacgtgtgctcttccgatcttggaggccccgctgggattcgaacccaggatctcctgtttgatcgtcggactgtagaactctgaac

SEQ ID NO: 183 - DNA, 87 bp, synthetic construct
  source 1..87: mol_type = other DNA
agacgtgtgctcttccgatcttggaggccccagcgagatttgaactcgcgacccctggtttgatcgtcggactgtagaactctgaac

SEQ ID NO: 184 - DNA, 87 bp, synthetic construct
  source 1..87: mol_type = other DNA
agacgtgtgctcttccgatcttggaggcacggacggggttcgaacccgtgatcttcggtttgatcgtcggactgtagaactctgaac

SEQ ID NO: 185 - DNA, 87 bp, synthetic construct
  source 1..87: mol_type = other DNA
agacgtgtgctcttccgatcttggtgaccccgacgtgatttgaacacgcaaccttctgatcgatcgtcggactgtagaactctgaac

SEQ ID NO: 186 - DNA, 87 bp, synthetic construct
  source 1..87: mol_type = other DNA
agacgtgtgctcttccgatcttggtccttcaagctggaatcgaaccagcaacctaaggaccgatcgtcggactgtagaactctgaac

SEQ ID NO: 187 - DNA, 87 bp, synthetic construct
  source 1..87: mol_type = other DNA
agacgtgtgctcttccgatcttggtccttcgagccggaatcgaaccagcgacctaaggatcgatcgtcggactgtagaactctgaac

SEQ ID NO: 188 - DNA, 87 bp, synthetic construct
  source 1..87: mol_type = other DNA
agacgtgtgctcttccgatcttggctctccaagtcggaatcaaaccagcacctaagaatctgatcgtcggactgtagaactctgaac

SEQ ID NO: 189 - DNA, 87 bp, synthetic construct
  source 1..87: mol_type = other DNA
agacgtgtgctcttccgatcttggtgtttccgcccggtttcgaaccggggacctttcgcgtgatcgtcggactgtagaactctgaac

SEQ ID NO: 190 - DNA, 87 bp, synthetic construct
  source 1..87: mol_type = other DNA
agacgtgtgctcttccgatcttggtggaagtgctggggatcgaacccagagcctcatgaatgatcgtcggactgtagaactctgaac

SEQ ID NO: 191 - DNA, 87 bp, synthetic construct
  source 1..87: mol_type = other DNA
agacgtgtgctcttccgatcttggtggttccactggggctcgaacccaggaccttctgcgtgatcgtcggactgtagaactctgaac

SEQ ID NO: 192 - DNA, 87 bp, synthetic construct
  source 1..87: mol_type = other DNA
agacgtgtgctcttccgatcttggtcagagtgttcattggtcatgaaatcttctgggtgtagatcgtcggactgtagaactctgaac

SEQ ID NO: 193 - DNA, 87 bp, synthetic construct
  source 1..87: mol_type = other DNA
agacgtgtgctcttccgatcttggtggtaaaaagaggatttaaacctctgtgtttagatttgatcgtcggactgtagaactctgaac

SEQ ID NO: 194 - DNA, 87 bp, synthetic construct
  source 1..87: mol_type = other DNA
agacgtgtgctcttccgatcttggcagaagttaaacttgtgtgttttcttagggctttgaagatcgtcggactgtagaactctgaac

SEQ ID NO: 195 - DNA, 87 bp, synthetic construct
  source 1..87: mol_type = other DNA
agacgtgtgctcttccgatcttggtgtcttgagaagagaagatcttcatttcaggtttacagatcgtcggactgtagaactctgaac

SEQ ID NO: 196 - DNA, 87 bp, synthetic construct
  source 1..87: mol_type = other DNA
agacgtgtgctcttccgatcttggtaagaaaggaaggaatcgaaccccctaaaattggtttgatcgtcggactgtagaactctgaac

SEQ ID NO: 197 - DNA, 87 bp, synthetic construct
  source 1..87: mol_type = other DNA
agacgtgtgctcttccgatcttggtaagaaagccatgtttttaaacatggaagcatgaattgatcgtcggactgtagaactctgaac

SEQ ID NO: 198 - DNA, 87 bp, synthetic construct
  source 1..87: mol_type = other DNA
agacgtgtgctcttccgatcttggtcaagaagaaggagctactccccaccaccagcacccagatcgtcggactgtagaactctgaac

SEQ ID NO: 199 - DNA, 87 bp, synthetic construct
  source 1..87: mol_type = other DNA
agacgtgtgctcttccgatcttggtgtttatgggatacaattatccatctaagcattttcagatcgtcggactgtagaactctgaac

SEQ ID NO: 200 - DNA, 87 bp, synthetic construct
  source 1..87: mol_type = other DNA
agacgtgtgctcttccgatcttggtagtacgggaaggatttaaaccaacgttttcggggtagatcgtcggactgtagaactctgaac

SEQ ID NO: 201 - DNA, 87 bp, synthetic construct
  source 1..87: mol_type = other DNA
agacgtgtgctcttccgatcttggtcactatggagattttaaggtctctaactttaacttagatcgtcggactgtagaactctgaac

SEQ ID NO: 202 - DNA, 87 bp, synthetic construct
  source 1..87: mol_type = other DNA
agacgtgtgctcttccgatcttggtattagggagaggatttgaacctctgggaacaaggttgatcgtcggactgtagaactctgaac

SEQ ID NO: 203 - DNA, 87 bp, synthetic construct
  source 1..87: mol_type = other DNA
agacgtgtgctcttccgatcttggtacttttatttggatttgcaccaaggtttttggttccgatcgtcggactgtagaactctgaac

SEQ ID NO: 204 - DNA, 87 bp, synthetic construct
  source 1..87: mol_type = other DNA
agacgtgtgctcttccgatcttggtagaaataagagggcttgaacctctataatttactctgatcgtcggactgtagaactctgaac

SEQ ID NO: 205 - DNA, 87 bp, synthetic construct
  source 1..87: mol_type = other DNA
agacgtgtgctcttccgatcttggggtgaataaggaggtttatttcctgttgtcagattcagatcgtcggactgtagaactctgaac

SEQ ID NO: 206 - DNA, 87 bp, synthetic construct
  source 1..87: mol_type = other DNA
agacgtgtgctcttccgatcttggtactctcttctgggtttattcagaatctactaattgggatcgtcggactgtagaactctgaac

SEQ ID NO: 207 - DNA, 87 bp, synthetic construct
  source 1..87: mol_type = other DNA
agacgtgtgctcttccgatcttggtatttctacacagcattcaactgcgaccaatgacatggatcgtcggactgtagaactctgaac

SEQ ID NO: 208 - DNA, 87 bp, synthetic construct
  source 1..87: mol_type = other DNA
agacgtgtgctcttccgatcttggctaggacaataggaattgaacctacacttaagaattcgatcgtcggactgtagaactctgaac

SEQ ID NO: 209 - DNA, 87 bp, synthetic construct
  source 1..87: mol_type = other DNA
agacgtgtgctcttccgatcttggaagtcttagtagagatttctctacaccttcgaatttggatcgtcggactgtagaactctgaac

SEQ ID NO: 210 - DNA, 87 bp, synthetic construct
  source 1..87: mol_type = other DNA
agacgtgtgctcttccgatcttggtaagatatatagattattgatctataatttaactttggatcgtcggactgtagaactctgaac

SEQ ID NO: 211 - DNA, 87 bp, synthetic construct
  source 1..87: mol_type = other DNA
agacgtgtgctcttccgatcttggctagattggcaggaattaaacctacgaaaatttagttgatcgtcggactgtagaactctgaac

SEQ ID NO: 212 - DNA, 87 bp, synthetic construct
  source 1..87: mol_type = other DNA
agacgtgtgctcttccgatcttggttggtaattatgaacatcatcataatctaatgagtcggatcgtcggactgtagaactctgaac

SEQ ID NO: 213 - DNA, 87 bp, synthetic construct
  source 1..87: mol_type = other DNA
agacgtgtgctcttccgatcttggtaaggactgtaagacttcatcctacatctattgaatggatcgtcggactgtagaactctgaac

SEQ ID NO: 214 - DNA, 87 bp, synthetic construct
  source 1..87: mol_type = other DNA
agacgtgtgctcttccgatcttggaaaaaaacctggagatcgaacccaggacctcatgcatgatcgtcggactgtagaactctgaac

SEQ ID NO: 215 - DNA, 87 bp, synthetic construct; identical to SEQ ID NO: 149
  source 1..87: mol_type = other DNA

SEQ ID NO: 216 - DNA, 87 bp, synthetic construct
  source 1..87: mol_type = other DNA
agacgtgtgctcttccgatcttggttccctgactaggattcaaacctgggccacggcggtggatcgtcggactgtagaactctgaac

SEQ ID NO: 217 - DNA, 87 bp, synthetic construct; identical to SEQ ID NO: 150
  source 1..87: mol_type = other DNA

SEQ ID NO: 218 - DNA, 87 bp, synthetic construct
  source 1..87: mol_type = other DNA
agacgtgtgctcttccgatcttggtaccccaggtgggactcgaacccacaatccctggcttgatcgtcggactgtagaactctgaac

SEQ ID NO: 219 - DNA, 87 bp, synthetic construct
  source 1..87: mol_type = other DNA
agacgtgtgctcttccgatcttggcgaccgcgccaggactcgaacctgcaatcttctgatcgatcgtcggactgtagaactctgaac

SEQ ID NO: 220 - DNA, 87 bp, synthetic construct
  source 1..87: mol_type = other DNA
agacgtgtgctcttccgatcttggcatctctgccgggactcgaacccagaacctctggattgatcgtcggactgtagaactctgaac

SEQ ID NO: 221 - DNA, 87 bp, synthetic construct; identical to SEQ ID NO: 154
  source 1..87: mol_type = other DNA

SEQ ID NO: 222 - DNA, 87 bp, synthetic construct; identical to SEQ ID NO: 155
  source 1..87: mol_type = other DNA

SEQ ID NO: 223 - DNA, 87 bp, synthetic construct; identical to SEQ ID NO: 156
  source 1..87: mol_type = other DNA

SEQ ID NO: 224 - DNA, 87 bp, synthetic construct; identical to SEQ ID NO: 157
  source 1..87: mol_type = other DNA

SEQ ID NO: 225 - DNA, 87 bp, synthetic construct; identical to SEQ ID NO: 158
  source 1..87: mol_type = other DNA

SEQ ID NO: 226 - DNA, 87 bp, synthetic construct; identical to SEQ ID NO: 159
  source 1..87: mol_type = other DNA

SEQ ID NO: 227 - DNA, 87 bp, synthetic construct; identical to SEQ ID NO: 160
  source 1..87: mol_type = other DNA

SEQ ID NO: 228 - DNA, 87 bp, synthetic construct
  source 1..87: mol_type = other DNA
agacgtgtgctcttccgatcttggttccctgaccaggaatcaaacctgggccatggaggtggatcgtcggactgtagaactctgaac

SEQ ID NO: 229 - DNA, 87 bp, synthetic construct; identical to SEQ ID NO: 162
  source 1..87: mol_type = other DNA

SEQ ID NO: 230 - DNA, 87 bp, synthetic construct; identical to SEQ ID NO: 163
  source 1..87: mol_type = other DNA

SEQ ID NO: 231 - DNA, 87 bp, synthetic construct
  source 1..87: mol_type = other DNA
agacgtgtgctcttccgatcttggtgtttccgcccggtttcgaaccggggacctttcgcttgatcgtcggactgtagaactctgaac

SEQ ID NO: 232 - DNA, 87 bp, synthetic construct; identical to SEQ ID NO: 165
  source 1..87: mol_type = other DNA

SEQ ID NO: 233 - DNA, 87 bp, synthetic construct; identical to SEQ ID NO: 166
  source 1..87: mol_type = other DNA

SEQ ID NO: 234 - DNA, 87 bp, synthetic construct
  source 1..87: mol_type = other DNA
agacgtgtgctcttccgatcttggtagttccactggggctcaaactcaggaccttctgcatgatcgtcggactgtagaactctgaac

SEQ ID NO: 235 - DNA, 87 bp, synthetic construct; identical to SEQ ID NO: 168
  source 1..87: mol_type = other DNA

SEQ ID NO: 236 - DNA, 87 bp, synthetic construct; identical to SEQ ID NO: 169
  source 1..87: mol_type = other DNA

SEQ ID NO: 237 - DNA, 87 bp, synthetic construct; identical to SEQ ID NO: 170
  source 1..87: mol_type = other DNA

SEQ ID NO: 238 - DNA, 87 bp, synthetic construct
  source 1..87: mol_type = other DNA
agacgtgtgctcttccgatcttggtactgggagtggggttcgaacccacgcaggcaccagcgatcgtcggactgtagaactctgaac

SEQ ID NO: 239 - DNA, 87 bp, synthetic construct
  source 1..87: mol_type = other DNA
agacgtgtgctcttccgatcttggtgcctaatatggggctcgaacccatgaccctgggattgatcgtcggactgtagaactctgaac

SEQ ID NO: 240 - DNA, 87 bp, synthetic construct; identical to SEQ ID NO: 173
  source 1..87: mol_type = other DNA

SEQ ID NO: 241 - DNA, 87 bp, synthetic construct
  source 1..87: mol_type = other DNA
agacgtgtgctcttccgatcttggtgccccgtgtgaggatcgaactcacgaccttcagattgatcgtcggactgtagaactctgaac

SEQ ID NO: 242 - DNA, 87 bp, synthetic construct; identical to SEQ ID NO: 175
  source 1..87: mol_type = other DNA

SEQ ID NO: 243 - DNA, 87 bp, synthetic construct; identical to SEQ ID NO: 176
  source 1..87: mol_type = other DNA

SEQ ID NO: 244 - DNA, 87 bp, synthetic construct; identical to SEQ ID NO: 177
  source 1..87: mol_type = other DNA

SEQ ID NO: 245 - DNA, 87 bp, synthetic construct; identical to SEQ ID NO: 178
  source 1..87: mol_type = other DNA

SEQ ID NO: 246 - DNA, 87 bp, synthetic construct; identical to SEQ ID NO: 179
  source 1..87: mol_type = other DNA

SEQ ID NO: 247 - DNA, 87 bp, synthetic construct; identical to SEQ ID NO: 180
  source 1..87: mol_type = other DNA

SEQ ID NO: 248 - DNA, 87 bp, synthetic construct
  source 1..87: mol_type = other DNA
agacgtgtgctcttccgatcttggtgccgaaacccgggatcaaaccagggacctttagatcgatcgtcggactgtagaactctgaac

SEQ ID NO: 249 - DNA, 87 bp, synthetic construct; identical to SEQ ID NO: 182
  source 1..87: mol_type = other DNA

SEQ ID NO: 250 - DNA, 87 bp, synthetic construct; identical to SEQ ID NO: 183
  source 1..87: mol_type = other DNA

SEQ ID NO: 251 - DNA, 87 bp, synthetic construct; identical to SEQ ID NO: 184
  source 1..87: mol_type = other DNA

SEQ ID NO: 252 - DNA, 87 bp, synthetic construct; identical to SEQ ID NO: 185
  source 1..87: mol_type = other DNA

SEQ ID NO: 253 - DNA, 87 bp, synthetic construct; identical to SEQ ID NO: 186
  source 1..87: mol_type = other DNA

SEQ ID NO: 254 - DNA, 87 bp, synthetic construct; identical to SEQ ID NO: 187
  source 1..87: mol_type = other DNA

SEQ ID NO: 255 - DNA, 87 bp, synthetic construct; identical to SEQ ID NO: 188
  source 1..87: mol_type = other DNA

SEQ ID NO: 256 - DNA, 87 bp, synthetic construct; identical to SEQ ID NO: 189
  source 1..87: mol_type = other DNA

SEQ ID NO: 257 - DNA, 87 bp, synthetic construct
  source 1..87: mol_type = other DNA
agacgtgtgctcttccgatcttggctatggtactgggaattgaacccaggacttttgcatggatcgtcggactgtagaactctgaac

SEQ ID NO: 258 - DNA, 87 bp, synthetic construct; identical to SEQ ID NO: 191
  source 1..87: mol_type = other DNA